European Patent Application EP 4 112 725 A1, published January 4, 2023. Title: GLUTAMATE-CYSTEINE LIGASE VARIANT AND METHOD OF PRODUCING GLUTATHIONE USING THE SAME. Applicant: CJ CheilJedang Corporation. The sequence listing filed with the application follows.

SEQUENCE LISTING (29 sequences)

SEQ ID NO: 1 - protein, 678 aa, Saccharomyces cerevisiae
MGLLALGTPLQWFESRTYNEHIRDEGIEQLLYIFQAAGKRDNDPLFWGDELEYMVVDFDDKERNSMLDVCHDKILTELNMEDSSLCEANDVSFHPEYGRYMLEATPASPYLNYVGSYVEVNMQKRRAIAEYKLSEYARQDSKNNLHVGSRSVPLTLTVFPRMGCPDFINIKDPWNHKNAASRSLFLPDEVINRHVRFPNLTASIRTRRGEKVCMNVPMYKDIATPETDDSIYDRDWFLPEDKEAKLASKPGFIYMDSMGFGMGCSCLQVTFQAPNINKARYLYDALVNFAPIMLAFSAAAPAFKGWLADQDVRWNVISGAVDDRTPKERGVAPLLPKYNKNGFGGIAKDVQDKVLEIPKSRYSSVDLFLGGSKFFNRTYNDTNVPINEKVLGRLLENDKAPLDYDLAKHFAHLYIRDPVSTFEELLNQDNKTSSNHFENIQSTNWQTLRFKPPTQQATPDKKDSPGWRVEFRPFEVQLLDFENAAYSVLIYLIVDSILTFSDNINAYIHMSKVWENMKIAHHRDAILFEKFHWKKSFRNDTDVETEDYSISEIFHNPENGIFPQFVTPILCQKGFVTKDWKELKHSSKHERLYYYLKLISDRASGELPTTAKFFRNFVLQHPDYKHDSKISKSINYDLLSTCDRLTHLDDSKGELTSFLGAEIAEYVKKNKPSIESKC

SEQ ID NO: 2 - DNA, 2037 bp, Saccharomyces cerevisiae
atgggactcttagctttgggcacgcctttgcagtggtttgagtctaggacgtacaatgaacacataagggatgaaggtatcgagcagttgttgtatattttccaagctgctggtaaaagagacaatgaccctcttttttggggagacgagcttgagtacatggttgtagattttgatgataaggagagaaattctatgctcgacgtttgccatgacaagatactcactgagcttaatatggaggattcgtccctttgtgaggctaacgatgtgagttttcaccctgagtatggccggtatatgttagaggcaacaccagcttctccatatttgaattacgtgggtagttacgttgaggttaacatgcaaaaaagacgtgccattgcagaatataagctatctgaatatgcgagacaagatagtaaaaataacttgcatgtgggctccaggtctgtccctttgacgctgactgtcttcccgaggatgggatgccccgactttattaacattaaggatccgtggaatcataaaaatgccgcttccaggtctctgtttttacccgatgaagtcattaacagacatgtcaggtttcctaacttgacagcatccatcaggaccaggcgtggtgaaaaagtttgcatgaatgttcccatgtataaagatatagctactccagaaacggatgactccatctacgatcgagattggtttttaccagaagacaaagaggcgaaactggcttccaaaccgggtttcatttatatggattccatgggttttggcatgggctgttcgtgcttacaagtgacctttcaggcacccaatatcaacaaggcacgttacctgtacgatgcattagtgaattttgcacctataatgctagccttctctgccgctgcgcctgcttttaaaggttggctagccgaccaagatgttcgttggaatgtgatatctggtgcggtggacgaccgtactccgaaggaaagaggtgttgcgccattactacccaaatacaacaagaacggatttggaggcattgccaaagacgtacaagataaagtccttgaaataccaaagtcaagatatagttcggttgatcttttcttgggtgggtcgaaatttttcaataggacttataacgacacaaatgtacctattaatgaaaaagtattaggacgactactagagaatgataaggcgccactggactatgatcttgctaaacattttgcgcatctctacataagagatccagtatctacattcgaagaactgttgaatcaggacaacaaaacgtcttcaaatcactttgaaaacatccaaagtacaaattggcagacattacgttttaaaccccccacacaacaagcaaccccggacaaaaaggattctcctggttggagagtggaattcagaccatttgaagtgcaactattagattttgagaacgctgcgtattccgtgctcatatacttgattgtcgatagcattttgaccttttccgataatattaacgcatatattcatatgtccaaagtatgggaaaatatgaagatagcccatcacagagatgctatcctatttgaaaaatttcattggaaaaaatcatttcgcaacgacaccgatgtggaaactgaagattattctataagcgagattttccataatccagagaatggtatatttcctcaatttgttacgccaatcctatgccaaaaagggtttgtaaccaaagattggaaagaattaaagcattcttccaaacacgagagactatactattatttaaagctaatttctgatagagcaagcggtgaattgccaacaacagcaaaattctttagaaattttgtactacaacatccagattacaaacatgattcaaaaatttcaaagtcgatcaattatgatttgctttctacgtgtgatagacttacccatttagacgattcaaaaggtgaattgacatcctttttaggagctgaaattgcagaatatgtaaaaaaaaataagccttcaatagaaagcaaatgttaa

SEQ ID NO: 3 - protein, 678 aa, Artificial Sequence
  S.cerevisiae GSH1 C86A
MGLLALGTPLQWFESRTYNEHIRDEGIEQLLYIFQAAGKRDNDPLFWGDELEYMVVDFDDKERNSMLDVCHDKILTELNMEDSSLAEANDVSFHPEYGRYMLEATPASPYLNYVGSYVEVNMQKRRAIAEYKLSEYARQDSKNNLHVGSRSVPLTLTVFPRMGCPDFINIKDPWNHKNAASRSLFLPDEVINRHVRFPNLTASIRTRRGEKVCMNVPMYKDIATPETDDSIYDRDWFLPEDKEAKLASKPGFIYMDSMGFGMGCSCLQVTFQAPNINKARYLYDALVNFAPIMLAFSAAAPAFKGWLADQDVRWNVISGAVDDRTPKERGVAPLLPKYNKNGFGGIAKDVQDKVLEIPKSRYSSVDLFLGGSKFFNRTYNDTNVPINEKVLGRLLENDKAPLDYDLAKHFAHLYIRDPVSTFEELLNQDNKTSSNHFENIQSTNWQTLRFKPPTQQATPDKKDSPGWRVEFRPFEVQLLDFENAAYSVLIYLIVDSILTFSDNINAYIHMSKVWENMKIAHHRDAILFEKFHWKKSFRNDTDVETEDYSISEIFHNPENGIFPQFVTPILCQKGFVTKDWKELKHSSKHERLYYYLKLISDRASGELPTTAKFFRNFVLQHPDYKHDSKISKSINYDLLSTCDRLTHLDDSKGELTSFLGAEIAEYVKKNKPSIESKC

SEQ ID NO: 4 - protein, 678 aa, Artificial Sequence
  S.cerevisiae GSH1 C86D
MGLLALGTPLQWFESRTYNEHIRDEGIEQLLYIFQAAGKRDNDPLFWGDELEYMVVDFDDKERNSMLDVCHDKILTELNMEDSSLDEANDVSFHPEYGRYMLEATPASPYLNYVGSYVEVNMQKRRAIAEYKLSEYARQDSKNNLHVGSRSVPLTLTVFPRMGCPDFINIKDPWNHKNAASRSLFLPDEVINRHVRFPNLTASIRTRRGEKVCMNVPMYKDIATPETDDSIYDRDWFLPEDKEAKLASKPGFIYMDSMGFGMGCSCLQVTFQAPNINKARYLYDALVNFAPIMLAFSAAAPAFKGWLADQDVRWNVISGAVDDRTPKERGVAPLLPKYNKNGFGGIAKDVQDKVLEIPKSRYSSVDLFLGGSKFFNRTYNDTNVPINEKVLGRLLENDKAPLDYDLAKHFAHLYIRDPVSTFEELLNQDNKTSSNHFENIQSTNWQTLRFKPPTQQATPDKKDSPGWRVEFRPFEVQLLDFENAAYSVLIYLIVDSILTFSDNINAYIHMSKVWENMKIAHHRDAILFEKFHWKKSFRNDTDVETEDYSISEIFHNPENGIFPQFVTPILCQKGFVTKDWKELKHSSKHERLYYYLKLISDRASGELPTTAKFFRNFVLQHPDYKHDSKISKSINYDLLSTCDRLTHLDDSKGELTSFLGAEIAEYVKKNKPSIESKC

SEQ ID NO: 5 - protein, 678 aa, Artificial Sequence
  S.cerevisiae GSH1 C86E
MGLLALGTPLQWFESRTYNEHIRDEGIEQLLYIFQAAGKRDNDPLFWGDELEYMVVDFDDKERNSMLDVCHDKILTELNMEDSSLEEANDVSFHPEYGRYMLEATPASPYLNYVGSYVEVNMQKRRAIAEYKLSEYARQDSKNNLHVGSRSVPLTLTVFPRMGCPDFINIKDPWNHKNAASRSLFLPDEVINRHVRFPNLTASIRTRRGEKVCMNVPMYKDIATPETDDSIYDRDWFLPEDKEAKLASKPGFIYMDSMGFGMGCSCLQVTFQAPNINKARYLYDALVNFAPIMLAFSAAAPAFKGWLADQDVRWNVISGAVDDRTPKERGVAPLLPKYNKNGFGGIAKDVQDKVLEIPKSRYSSVDLFLGGSKFFNRTYNDTNVPINEKVLGRLLENDKAPLDYDLAKHFAHLYIRDPVSTFEELLNQDNKTSSNHFENIQSTNWQTLRFKPPTQQATPDKKDSPGWRVEFRPFEVQLLDFENAAYSVLIYLIVDSILTFSDNINAYIHMSKVWENMKIAHHRDAILFEKFHWKKSFRNDTDVETEDYSISEIFHNPENGIFPQFVTPILCQKGFVTKDWKELKHSSKHERLYYYLKLISDRASGELPTTAKFFRNFVLQHPDYKHDSKISKSINYDLLSTCDRLTHLDDSKGELTSFLGAEIAEYVKKNKPSIESKC

SEQ ID NO: 6 - protein, 678 aa, Artificial Sequence
  S.cerevisiae GSH1 C86F
MGLLALGTPLQWFESRTYNEHIRDEGIEQLLYIFQAAGKRDNDPLFWGDELEYMVVDFDDKERNSMLDVCHDKILTELNMEDSSLFEANDVSFHPEYGRYMLEATPASPYLNYVGSYVEVNMQKRRAIAEYKLSEYARQDSKNNLHVGSRSVPLTLTVFPRMGCPDFINIKDPWNHKNAASRSLFLPDEVINRHVRFPNLTASIRTRRGEKVCMNVPMYKDIATPETDDSIYDRDWFLPEDKEAKLASKPGFIYMDSMGFGMGCSCLQVTFQAPNINKARYLYDALVNFAPIMLAFSAAAPAFKGWLADQDVRWNVISGAVDDRTPKERGVAPLLPKYNKNGFGGIAKDVQDKVLEIPKSRYSSVDLFLGGSKFFNRTYNDTNVPINEKVLGRLLENDKAPLDYDLAKHFAHLYIRDPVSTFEELLNQDNKTSSNHFENIQSTNWQTLRFKPPTQQATPDKKDSPGWRVEFRPFEVQLLDFENAAYSVLIYLIVDSILTFSDNINAYIHMSKVWENMKIAHHRDAILFEKFHWKKSFRNDTDVETEDYSISEIFHNPENGIFPQFVTPILCQKGFVTKDWKELKHSSKHERLYYYLKLISDRASGELPTTAKFFRNFVLQHPDYKHDSKISKSINYDLLSTCDRLTHLDDSKGELTSFLGAEIAEYVKKNKPSIESKC

SEQ ID NO: 7 - protein, 678 aa, Artificial Sequence
  S.cerevisiae GSH1 C86G
MGLLALGTPLQWFESRTYNEHIRDEGIEQLLYIFQAAGKRDNDPLFWGDELEYMVVDFDDKERNSMLDVCHDKILTELNMEDSSLGEANDVSFHPEYGRYMLEATPASPYLNYVGSYVEVNMQKRRAIAEYKLSEYARQDSKNNLHVGSRSVPLTLTVFPRMGCPDFINIKDPWNHKNAASRSLFLPDEVINRHVRFPNLTASIRTRRGEKVCMNVPMYKDIATPETDDSIYDRDWFLPEDKEAKLASKPGFIYMDSMGFGMGCSCLQVTFQAPNINKARYLYDALVNFAPIMLAFSAAAPAFKGWLADQDVRWNVISGAVDDRTPKERGVAPLLPKYNKNGFGGIAKDVQDKVLEIPKSRYSSVDLFLGGSKFFNRTYNDTNVPINEKVLGRLLENDKAPLDYDLAKHFAHLYIRDPVSTFEELLNQDNKTSSNHFENIQSTNWQTLRFKPPTQQATPDKKDSPGWRVEFRPFEVQLLDFENAAYSVLIYLIVDSILTFSDNINAYIHMSKVWENMKIAHHRDAILFEKFHWKKSFRNDTDVETEDYSISEIFHNPENGIFPQFVTPILCQKGFVTKDWKELKHSSKHERLYYYLKLISDRASGELPTTAKFFRNFVLQHPDYKHDSKISKSINYDLLSTCDRLTHLDDSKGELTSFLGAEIAEYVKKNKPSIESKC

SEQ ID NO: 8 - protein, 678 aa, Artificial Sequence
  S.cerevisiae GSH1 C86H
MGLLALGTPLQWFESRTYNEHIRDEGIEQLLYIFQAAGKRDNDPLFWGDELEYMVVDFDDKERNSMLDVCHDKILTELNMEDSSLHEANDVSFHPEYGRYMLEATPASPYLNYVGSYVEVNMQKRRAIAEYKLSEYARQDSKNNLHVGSRSVPLTLTVFPRMGCPDFINIKDPWNHKNAASRSLFLPDEVINRHVRFPNLTASIRTRRGEKVCMNVPMYKDIATPETDDSIYDRDWFLPEDKEAKLASKPGFIYMDSMGFGMGCSCLQVTFQAPNINKARYLYDALVNFAPIMLAFSAAAPAFKGWLADQDVRWNVISGAVDDRTPKERGVAPLLPKYNKNGFGGIAKDVQDKVLEIPKSRYSSVDLFLGGSKFFNRTYNDTNVPINEKVLGRLLENDKAPLDYDLAKHFAHLYIRDPVSTFEELLNQDNKTSSNHFENIQSTNWQTLRFKPPTQQATPDKKDSPGWRVEFRPFEVQLLDFENAAYSVLIYLIVDSILTFSDNINAYIHMSKVWENMKIAHHRDAILFEKFHWKKSFRNDTDVETEDYSISEIFHNPENGIFPQFVTPILCQKGFVTKDWKELKHSSKHERLYYYLKLISDRASGELPTTAKFFRNFVLQHPDYKHDSKISKSINYDLLSTCDRLTHLDDSKGELTSFLGAEIAEYVKKNKPSIESKC

SEQ ID NO: 9 - protein, 678 aa, Artificial Sequence
  S.cerevisiae GSH1 C86I
MGLLALGTPLQWFESRTYNEHIRDEGIEQLLYIFQAAGKRDNDPLFWGDELEYMVVDFDDKERNSMLDVCHDKILTELNMEDSSLIEANDVSFHPEYGRYMLEATPASPYLNYVGSYVEVNMQKRRAIAEYKLSEYARQDSKNNLHVGSRSVPLTLTVFPRMGCPDFINIKDPWNHKNAASRSLFLPDEVINRHVRFPNLTASIRTRRGEKVCMNVPMYKDIATPETDDSIYDRDWFLPEDKEAKLASKPGFIYMDSMGFGMGCSCLQVTFQAPNINKARYLYDALVNFAPIMLAFSAAAPAFKGWLADQDVRWNVISGAVDDRTPKERGVAPLLPKYNKNGFGGIAKDVQDKVLEIPKSRYSSVDLFLGGSKFFNRTYNDTNVPINEKVLGRLLENDKAPLDYDLAKHFAHLYIRDPVSTFEELLNQDNKTSSNHFENIQSTNWQTLRFKPPTQQATPDKKDSPGWRVEFRPFEVQLLDFENAAYSVLIYLIVDSILTFSDNINAYIHMSKVWENMKIAHHRDAILFEKFHWKKSFRNDTDVETEDYSISEIFHNPENGIFPQFVTPILCQKGFVTKDWKELKHSSKHERLYYYLKLISDRASGELPTTAKFFRNFVLQHPDYKHDSKISKSINYDLLSTCDRLTHLDDSKGELTSFLGAEIAEYVKKNKPSIESKC

SEQ ID NO: 10 - protein, 678 aa, Artificial Sequence
  S.cerevisiae GSH1 C86K
MGLLALGTPLQWFESRTYNEHIRDEGIEQLLYIFQAAGKRDNDPLFWGDELEYMVVDFDDKERNSMLDVCHDKILTELNMEDSSLKEANDVSFHPEYGRYMLEATPASPYLNYVGSYVEVNMQKRRAIAEYKLSEYARQDSKNNLHVGSRSVPLTLTVFPRMGCPDFINIKDPWNHKNAASRSLFLPDEVINRHVRFPNLTASIRTRRGEKVCMNVPMYKDIATPETDDSIYDRDWFLPEDKEAKLASKPGFIYMDSMGFGMGCSCLQVTFQAPNINKARYLYDALVNFAPIMLAFSAAAPAFKGWLADQDVRWNVISGAVDDRTPKERGVAPLLPKYNKNGFGGIAKDVQDKVLEIPKSRYSSVDLFLGGSKFFNRTYNDTNVPINEKVLGRLLENDKAPLDYDLAKHFAHLYIRDPVSTFEELLNQDNKTSSNHFENIQSTNWQTLRFKPPTQQATPDKKDSPGWRVEFRPFEVQLLDFENAAYSVLIYLIVDSILTFSDNINAYIHMSKVWENMKIAHHRDAILFEKFHWKKSFRNDTDVETEDYSISEIFHNPENGIFPQFVTPILCQKGFVTKDWKELKHSSKHERLYYYLKLISDRASGELPTTAKFFRNFVLQHPDYKHDSKISKSINYDLLSTCDRLTHLDDSKGELTSFLGAEIAEYVKKNKPSIESKC

SEQ ID NO: 11 - protein, 678 aa, Artificial Sequence
  S.cerevisiae GSH1 C86L
MGLLALGTPLQWFESRTYNEHIRDEGIEQLLYIFQAAGKRDNDPLFWGDELEYMVVDFDDKERNSMLDVCHDKILTELNMEDSSLLEANDVSFHPEYGRYMLEATPASPYLNYVGSYVEVNMQKRRAIAEYKLSEYARQDSKNNLHVGSRSVPLTLTVFPRMGCPDFINIKDPWNHKNAASRSLFLPDEVINRHVRFPNLTASIRTRRGEKVCMNVPMYKDIATPETDDSIYDRDWFLPEDKEAKLASKPGFIYMDSMGFGMGCSCLQVTFQAPNINKARYLYDALVNFAPIMLAFSAAAPAFKGWLADQDVRWNVISGAVDDRTPKERGVAPLLPKYNKNGFGGIAKDVQDKVLEIPKSRYSSVDLFLGGSKFFNRTYNDTNVPINEKVLGRLLENDKAPLDYDLAKHFAHLYIRDPVSTFEELLNQDNKTSSNHFENIQSTNWQTLRFKPPTQQATPDKKDSPGWRVEFRPFEVQLLDFENAAYSVLIYLIVDSILTFSDNINAYIHMSKVWENMKIAHHRDAILFEKFHWKKSFRNDTDVETEDYSISEIFHNPENGIFPQFVTPILCQKGFVTKDWKELKHSSKHERLYYYLKLISDRASGELPTTAKFFRNFVLQHPDYKHDSKISKSINYDLLSTCDRLTHLDDSKGELTSFLGAEIAEYVKKNKPSIESKC

SEQ ID NO: 12 - protein, 678 aa, Artificial Sequence
  S.cerevisiae GSH1 C86M
MGLLALGTPLQWFESRTYNEHIRDEGIEQLLYIFQAAGKRDNDPLFWGDELEYMVVDFDDKERNSMLDVCHDKILTELNMEDSSLMEANDVSFHPEYGRYMLEATPASPYLNYVGSYVEVNMQKRRAIAEYKLSEYARQDSKNNLHVGSRSVPLTLTVFPRMGCPDFINIKDPWNHKNAASRSLFLPDEVINRHVRFPNLTASIRTRRGEKVCMNVPMYKDIATPETDDSIYDRDWFLPEDKEAKLASKPGFIYMDSMGFGMGCSCLQVTFQAPNINKARYLYDALVNFAPIMLAFSAAAPAFKGWLADQDVRWNVISGAVDDRTPKERGVAPLLPKYNKNGFGGIAKDVQDKVLEIPKSRYSSVDLFLGGSKFFNRTYNDTNVPINEKVLGRLLENDKAPLDYDLAKHFAHLYIRDPVSTFEELLNQDNKTSSNHFENIQSTNWQTLRFKPPTQQATPDKKDSPGWRVEFRPFEVQLLDFENAAYSVLIYLIVDSILTFSDNINAYIHMSKVWENMKIAHHRDAILFEKFHWKKSFRNDTDVETEDYSISEIFHNPENGIFPQFVTPILCQKGFVTKDWKELKHSSKHERLYYYLKLISDRASGELPTTAKFFRNFVLQHPDYKHDSKISKSINYDLLSTCDRLTHLDDSKGELTSFLGAEIAEYVKKNKPSIESKC

SEQ ID NO: 13 - protein, 678 aa, Artificial Sequence
  S.cerevisiae GSH1 C86N
MGLLALGTPLQWFESRTYNEHIRDEGIEQLLYIFQAAGKRDNDPLFWGDELEYMVVDFDDKERNSMLDVCHDKILTELNMEDSSLNEANDVSFHPEYGRYMLEATPASPYLNYVGSYVEVNMQKRRAIAEYKLSEYARQDSKNNLHVGSRSVPLTLTVFPRMGCPDFINIKDPWNHKNAASRSLFLPDEVINRHVRFPNLTASIRTRRGEKVCMNVPMYKDIATPETDDSIYDRDWFLPEDKEAKLASKPGFIYMDSMGFGMGCSCLQVTFQAPNINKARYLYDALVNFAPIMLAFSAAAPAFKGWLADQDVRWNVISGAVDDRTPKERGVAPLLPKYNKNGFGGIAKDVQDKVLEIPKSRYSSVDLFLGGSKFFNRTYNDTNVPINEKVLGRLLENDKAPLDYDLAKHFAHLYIRDPVSTFEELLNQDNKTSSNHFENIQSTNWQTLRFKPPTQQATPDKKDSPGWRVEFRPFEVQLLDFENAAYSVLIYLIVDSILTFSDNINAYIHMSKVWENMKIAHHRDAILFEKFHWKKSFRNDTDVETEDYSISEIFHNPENGIFPQFVTPILCQKGFVTKDWKELKHSSKHERLYYYLKLISDRASGELPTTAKFFRNFVLQHPDYKHDSKISKSINYDLLSTCDRLTHLDDSKGELTSFLGAEIAEYVKKNKPSIESKC

SEQ ID NO: 14 - protein, 678 aa, Artificial Sequence
  S.cerevisiae GSH1 C86P
MGLLALGTPLQWFESRTYNEHIRDEGIEQLLYIFQAAGKRDNDPLFWGDELEYMVVDFDDKERNSMLDVCHDKILTELNMEDSSLPEANDVSFHPEYGRYMLEATPASPYLNYVGSYVEVNMQKRRAIAEYKLSEYARQDSKNNLHVGSRSVPLTLTVFPRMGCPDFINIKDPWNHKNAASRSLFLPDEVINRHVRFPNLTASIRTRRGEKVCMNVPMYKDIATPETDDSIYDRDWFLPEDKEAKLASKPGFIYMDSMGFGMGCSCLQVTFQAPNINKARYLYDALVNFAPIMLAFSAAAPAFKGWLADQDVRWNVISGAVDDRTPKERGVAPLLPKYNKNGFGGIAKDVQDKVLEIPKSRYSSVDLFLGGSKFFNRTYNDTNVPINEKVLGRLLENDKAPLDYDLAKHFAHLYIRDPVSTFEELLNQDNKTSSNHFENIQSTNWQTLRFKPPTQQATPDKKDSPGWRVEFRPFEVQLLDFENAAYSVLIYLIVDSILTFSDNINAYIHMSKVWENMKIAHHRDAILFEKFHWKKSFRNDTDVETEDYSISEIFHNPENGIFPQFVTPILCQKGFVTKDWKELKHSSKHERLYYYLKLISDRASGELPTTAKFFRNFVLQHPDYKHDSKISKSINYDLLSTCDRLTHLDDSKGELTSFLGAEIAEYVKKNKPSIESKC

SEQ ID NO: 15 - protein, 678 aa, Artificial Sequence
  S.cerevisiae GSH1 C86Q
MGLLALGTPLQWFESRTYNEHIRDEGIEQLLYIFQAAGKRDNDPLFWGDELEYMVVDFDDKERNSMLDVCHDKILTELNMEDSSLQEANDVSFHPEYGRYMLEATPASPYLNYVGSYVEVNMQKRRAIAEYKLSEYARQDSKNNLHVGSRSVPLTLTVFPRMGCPDFINIKDPWNHKNAASRSLFLPDEVINRHVRFPNLTASIRTRRGEKVCMNVPMYKDIATPETDDSIYDRDWFLPEDKEAKLASKPGFIYMDSMGFGMGCSCLQVTFQAPNINKARYLYDALVNFAPIMLAFSAAAPAFKGWLADQDVRWNVISGAVDDRTPKERGVAPLLPKYNKNGFGGIAKDVQDKVLEIPKSRYSSVDLFLGGSKFFNRTYNDTNVPINEKVLGRLLENDKAPLDYDLAKHFAHLYIRDPVSTFEELLNQDNKTSSNHFENIQSTNWQTLRFKPPTQQATPDKKDSPGWRVEFRPFEVQLLDFENAAYSVLIYLIVDSILTFSDNINAYIHMSKVWENMKIAHHRDAILFEKFHWKKSFRNDTDVETEDYSISEIFHNPENGIFPQFVTPILCQKGFVTKDWKELKHSSKHERLYYYLKLISDRASGELPTTAKFFRNFVLQHPDYKHDSKISKSINYDLLSTCDRLTHLDDSKGELTSFLGAEIAEYVKKNKPSIESKC

SEQ ID NO: 16 - protein, 678 aa, Artificial Sequence
  S.cerevisiae GSH1 C86R
MGLLALGTPLQWFESRTYNEHIRDEGIEQLLYIFQAAGKRDNDPLFWGDELEYMVVDFDDKERNSMLDVCHDKILTELNMEDSSLREANDVSFHPEYGRYMLEATPASPYLNYVGSYVEVNMQKRRAIAEYKLSEYARQDSKNNLHVGSRSVPLTLTVFPRMGCPDFINIKDPWNHKNAASRSLFLPDEVINRHVRFPNLTASIRTRRGEKVCMNVPMYKDIATPETDDSIYDRDWFLPEDKEAKLASKPGFIYMDSMGFGMGCSCLQVTFQAPNINKARYLYDALVNFAPIMLAFSAAAPAFKGWLADQDVRWNVISGAVDDRTPKERGVAPLLPKYNKNGFGGIAKDVQDKVLEIPKSRYSSVDLFLGGSKFFNRTYNDTNVPINEKVLGRLLENDKAPLDYDLAKHFAHLYIRDPVSTFEELLNQDNKTSSNHFENIQSTNWQTLRFKPPTQQATPDKKDSPGWRVEFRPFEVQLLDFENAAYSVLIYLIVDSILTFSDNINAYIHMSKVWENMKIAHHRDAILFEKFHWKKSFRNDTDVETEDYSISEIFHNPENGIFPQFVTPILCQKGFVTKDWKELKHSSKHERLYYYLKLISDRASGELPTTAKFFRNFVLQHPDYKHDSKISKSINYDLLSTCDRLTHLDDSKGELTSFLGAEIAEYVKKNKPSIESKC

SEQ ID NO: 17 - protein, 678 aa, Artificial Sequence
  S.cerevisiae GSH1 C86S
MGLLALGTPLQWFESRTYNEHIRDEGIEQLLYIFQAAGKRDNDPLFWGDELEYMVVDFDDKERNSMLDVCHDKILTELNMEDSSLSEANDVSFHPEYGRYMLEATPASPYLNYVGSYVEVNMQKRRAIAEYKLSEYARQDSKNNLHVGSRSVPLTLTVFPRMGCPDFINIKDPWNHKNAASRSLFLPDEVINRHVRFPNLTASIRTRRGEKVCMNVPMYKDIATPETDDSIYDRDWFLPEDKEAKLASKPGFIYMDSMGFGMGCSCLQVTFQAPNINKARYLYDALVNFAPIMLAFSAAAPAFKGWLADQDVRWNVISGAVDDRTPKERGVAPLLPKYNKNGFGGIAKDVQDKVLEIPKSRYSSVDLFLGGSKFFNRTYNDTNVPINEKVLGRLLENDKAPLDYDLAKHFAHLYIRDPVSTFEELLNQDNKTSSNHFENIQSTNWQTLRFKPPTQQATPDKKDSPGWRVEFRPFEVQLLDFENAAYSVLIYLIVDSILTFSDNINAYIHMSKVWENMKIAHHRDAILFEKFHWKKSFRNDTDVETEDYSISEIFHNPENGIFPQFVTPILCQKGFVTKDWKELKHSSKHERLYYYLKLISDRASGELPTTAKFFRNFVLQHPDYKHDSKISKSINYDLLSTCDRLTHLDDSKGELTSFLGAEIAEYVKKNKPSIESKC

SEQ ID NO: 18 - protein, 678 aa, Artificial Sequence
  S.cerevisiae GSH1 C86T
MGLLALGTPLQWFESRTYNEHIRDEGIEQLLYIFQAAGKRDNDPLFWGDELEYMVVDFDDKERNSMLDVCHDKILTELNMEDSSLTEANDVSFHPEYGRYMLEATPASPYLNYVGSYVEVNMQKRRAIAEYKLSEYARQDSKNNLHVGSRSVPLTLTVFPRMGCPDFINIKDPWNHKNAASRSLFLPDEVINRHVRFPNLTASIRTRRGEKVCMNVPMYKDIATPETDDSIYDRDWFLPEDKEAKLASKPGFIYMDSMGFGMGCSCLQVTFQAPNINKARYLYDALVNFAPIMLAFSAAAPAFKGWLADQDVRWNVISGAVDDRTPKERGVAPLLPKYNKNGFGGIAKDVQDKVLEIPKSRYSSVDLFLGGSKFFNRTYNDTNVPINEKVLGRLLENDKAPLDYDLAKHFAHLYIRDPVSTFEELLNQDNKTSSNHFENIQSTNWQTLRFKPPTQQATPDKKDSPGWRVEFRPFEVQLLDFENAAYSVLIYLIVDSILTFSDNINAYIHMSKVWENMKIAHHRDAILFEKFHWKKSFRNDTDVETEDYSISEIFHNPENGIFPQFVTPILCQKGFVTKDWKELKHSSKHERLYYYLKLISDRASGELPTTAKFFRNFVLQHPDYKHDSKISKSINYDLLSTCDRLTHLDDSKGELTSFLGAEIAEYVKKNKPSIESKC

SEQ ID NO: 19 - protein, 678 aa, Artificial Sequence
  S.cerevisiae GSH1 C86V
MGLLALGTPLQWFESRTYNEHIRDEGIEQLLYIFQAAGKRDNDPLFWGDELEYMVVDFDDKERNSMLDVCHDKILTELNMEDSSLVEANDVSFHPEYGRYMLEATPASPYLNYVGSYVEVNMQKRRAIAEYKLSEYARQDSKNNLHVGSRSVPLTLTVFPRMGCPDFINIKDPWNHKNAASRSLFLPDEVINRHVRFPNLTASIRTRRGEKVCMNVPMYKDIATPETDDSIYDRDWFLPEDKEAKLASKPGFIYMDSMGFGMGCSCLQVTFQAPNINKARYLYDALVNFAPIMLAFSAAAPAFKGWLADQDVRWNVISGAVDDRTPKERGVAPLLPKYNKNGFGGIAKDVQDKVLEIPKSRYSSVDLFLGGSKFFNRTYNDTNVPINEKVLGRLLENDKAPLDYDLAKHFAHLYIRDPVSTFEELLNQDNKTSSNHFENIQSTNWQTLRFKPPTQQATPDKKDSPGWRVEFRPFEVQLLDFENAAYSVLIYLIVDSILTFSDNINAYIHMSKVWENMKIAHHRDAILFEKFHWKKSFRNDTDVETEDYSISEIFHNPENGIFPQFVTPILCQKGFVTKDWKELKHSSKHERLYYYLKLISDRASGELPTTAKFFRNFVLQHPDYKHDSKISKSINYDLLSTCDRLTHLDDSKGELTSFLGAEIAEYVKKNKPSIESKC

SEQ ID NO: 20 - protein, 678 aa, Artificial Sequence
  S.cerevisiae GSH1 C86W
MGLLALGTPLQWFESRTYNEHIRDEGIEQLLYIFQAAGKRDNDPLFWGDELEYMVVDFDDKERNSMLDVCHDKILTELNMEDSSLWEANDVSFHPEYGRYMLEATPASPYLNYVGSYVEVNMQKRRAIAEYKLSEYARQDSKNNLHVGSRSVPLTLTVFPRMGCPDFINIKDPWNHKNAASRSLFLPDEVINRHVRFPNLTASIRTRRGEKVCMNVPMYKDIATPETDDSIYDRDWFLPEDKEAKLASKPGFIYMDSMGFGMGCSCLQVTFQAPNINKARYLYDALVNFAPIMLAFSAAAPAFKGWLADQDVRWNVISGAVDDRTPKERGVAPLLPKYNKNGFGGIAKDVQDKVLEIPKSRYSSVDLFLGGSKFFNRTYNDTNVPINEKVLGRLLENDKAPLDYDLAKHFAHLYIRDPVSTFEELLNQDNKTSSNHFENIQSTNWQTLRFKPPTQQATPDKKDSPGWRVEFRPFEVQLLDFENAAYSVLIYLIVDSILTFSDNINAYIHMSKVWENMKIAHHRDAILFEKFHWKKSFRNDTDVETEDYSISEIFHNPENGIFPQFVTPILCQKGFVTKDWKELKHSSKHERLYYYLKLISDRASGELPTTAKFFRNFVLQHPDYKHDSKISKSINYDLLSTCDRLTHLDDSKGELTSFLGAEIAEYVKKNKPSIESKC

SEQ ID NO: 21 - protein, 678 aa, Artificial Sequence
  S.cerevisiae GSH1 C86Y
MGLLALGTPLQWFESRTYNEHIRDEGIEQLLYIFQAAGKRDNDPLFWGDELEYMVVDFDDKERNSMLDVCHDKILTELNMEDSSLYEANDVSFHPEYGRYMLEATPASPYLNYVGSYVEVNMQKRRAIAEYKLSEYARQDSKNNLHVGSRSVPLTLTVFPRMGCPDFINIKDPWNHKNAASRSLFLPDEVINRHVRFPNLTASIRTRRGEKVCMNVPMYKDIATPETDDSIYDRDWFLPEDKEAKLASKPGFIYMDSMGFGMGCSCLQVTFQAPNINKARYLYDALVNFAPIMLAFSAAAPAFKGWLADQDVRWNVISGAVDDRTPKERGVAPLLPKYNKNGFGGIAKDVQDKVLEIPKSRYSSVDLFLGGSKFFNRTYNDTNVPINEKVLGRLLENDKAPLDYDLAKHFAHLYIRDPVSTFEELLNQDNKTSSNHFENIQSTNWQTLRFKPPTQQATPDKKDSPGWRVEFRPFEVQLLDFENAAYSVLIYLIVDSILTFSDNINAYIHMSKVWENMKIAHHRDAILFEKFHWKKSFRNDTDVETEDYSISEIFHNPENGIFPQFVTPILCQKGFVTKDWKELKHSSKHERLYYYLKLISDRASGELPTTAKFFRNFVLQHPDYKHDSKISKSINYDLLSTCDRLTHLDDSKGELTSFLGAEIAEYVKKNKPSIESKC

SEQ ID NO: 22 - DNA, 33 bp, Artificial Sequence
  F_BamHI_GSH1
ggtaggatccatgggactcttagctttgggcac

SEQ ID NO: 23 - DNA, 25 bp, Artificial Sequence
  R_GSH1_C86R
ttagcctccctaagggacgaatcct

SEQ ID NO: 24 - DNA, 25 bp, Artificial Sequence
  F_GSH1_C86R
cgtcccttagggaggctaacgatgt

SEQ ID NO: 25 - DNA, 35 bp, Artificial Sequence
  R_XhoI_GSH1
atgactcgagttaacatttgctttctattgaaggc

SEQ ID NO: 26 - DNA, 33 bp, Artificial Sequence
  F_SpeI_GSH1_DW
tagaactagtactccttttatttcggttgtgaa

SEQ ID NO: 27 - DNA, 35 bp, Artificial Sequence
  R_NcoI_GSH1_DW
gctgccatgggaatagtgtgaaccgataactgtgt

SEQ ID NO: 28 - DNA, 27 bp, Artificial Sequence
  R_AL killer
gagcaatgaacccaataacgaaatctt

SEQ ID NO: 29 - DNA, 24 bp, Artificial Sequence
  F_BR killer
cttgacgttcgttcgactgatgag